European Patent Application EP 4 512 901 A1, published February 26, 2025. Title: A microorganism having gluconate repressor protein activity weakened and a method for producing L-arginine using the same. Applicant: 씨제이제일제당 (주). The sequence listing filed with the application follows.

SEQUENCE LISTING (38 sequences)

SEQ ID NO: 1 - protein, 250 aa, unidentified
  REGION 1..250: note = gluconate repressor
MPPANESPMTNPLGSAPTPAKPLLDSVLDELGQDIISGKVAVGDTFKLMDIGERFGISRTVAREAMRALEQLGLVASSRRIGITVLPQEEWAVFDKSIIRWRLNDEGQREGQLQSLTELRIAIEPIAARSVALHASTAELEKIRALATEMRQLGESGQGASQRFLEADVTFHELILRYCHNEMFAALIPSISAVLVGRTELGLQPDLPAHEALDNHDKLADALLNRDADAAETASRNILNEVRSALGTLN

SEQ ID NO: 2 - DNA, 753 bp, unidentified
  misc_feature 1..753: note = gluconate repressor
  source 1..753: mol_type = genomic DNA
atgcccccagcaaacgaaagtcctatgactaatccattaggttctgcccccaccccagccaagccacttcttgacagtgttcttgatgagctcggtcaagatatcatcagtggcaaggttgctgtcggagataccttcaagctgatggacatcggcgagcgttttggtatttcccgcacagtggcacgcgaagcaatgcgcgctttggagcagctcggtcttgtcgcttcttcacgtcgcattggcattactgttttgccacaggaagagtgggctgtttttgataagtccatcattcgctggcgtctcaatgacgaaggtcagcgtgaaggccagcttcagtctcttaccgagcttcgtattgctattgaaccgattgccgcgcgcagcgttgctcttcacgcgtcaaccgccgagctcgagaaaatccgcgcgctggcaacagagatgcgtcagttgggtgaatctggtcagggtgcgtcccagcgcttcctcgaagcggacgtcaccttccacgagctcatcttgcgttattgccacaatgagatgttcgctgcactgattccgtcgattagcgcggttcttgtcggccgcaccgagctcggcctgcagcctgatctgccggcgcacgaggcgctagacaaccacgataagcttgccgacgccctccttaaccgcgacgccgacgccgcagaaactgcgtcccgaaacatcctcaatgaggtgcgcagcgcgctgggcacgctgaactaa

SEQ ID NO: 3 - DNA, 34 bp, synthetic construct
  misc_feature 1..34: note = primer
  source 1..34: mol_type = other DNA
tcggtacccggggatccaagcaaccgtcggcgag

SEQ ID NO: 4 - DNA, 34 bp, synthetic construct
  misc_feature 1..34: note = primer
  source 1..34: mol_type = other DNA
tgcaggtcgactctagatttcgggacgcagtttc

SEQ ID NO: 5 - DNA, 34 bp, synthetic construct
  misc_feature 1..34: note = primer
  source 1..34: mol_type = other DNA
agcaaccttgccactgttgatatcttgaccgagc

SEQ ID NO: 6 - DNA, 35 bp, synthetic construct
  misc_feature 1..35: note = primer
  source 1..35: mol_type = other DNA
acagtggcaaggttgctgtcggagataccttcaag

SEQ ID NO: 7 - DNA, 33 bp, synthetic construct
  misc_feature 1..33: note = primer
  source 1..33: mol_type = other DNA
tcgcgtgccactgtggcggaaataccaaaacgc

SEQ ID NO: 8 - DNA, 33 bp, synthetic construct
  misc_feature 1..33: note = primer
  source 1..33: mol_type = other DNA
gccacagtggcacgcgaagcaatgcgcgctttg

SEQ ID NO: 9 - DNA, 35 bp, synthetic construct
  misc_feature 1..35: note = primer
  source 1..35: mol_type = other DNA
gcttcgcgtgccactaggcgggaaataccaaaacg

SEQ ID NO: 10 - DNA, 35 bp, synthetic construct
  misc_feature 1..35: note = primer
  source 1..35: mol_type = other DNA
ctagtggcacgcgaagcaatgcgcgctttggagca

SEQ ID NO: 11 - DNA, 31 bp, synthetic construct
  misc_feature 1..31: note = primer
  source 1..31: mol_type = other DNA
gcgcgcattgcttcggctgccactgtgcggg

SEQ ID NO: 12 - DNA, 34 bp, synthetic construct
  misc_feature 1..34: note = primer
  source 1..34: mol_type = other DNA
gccgaagcaatgcgcgctttggagcagctcggtc

SEQ ID NO: 13 - DNA, 35 bp, synthetic construct
  misc_feature 1..35: note = primer
  source 1..35: mol_type = other DNA
gtaatgccaatgcgagctgaagaagcgacaagacc

SEQ ID NO: 14 - DNA, 34 bp, synthetic construct
  misc_feature 1..34: note = primer
  source 1..34: mol_type = other DNA
gctcgcattggcattactgttttgccacaggaag

SEQ ID NO: 15 - DNA, 33 bp, synthetic construct
  misc_feature 1..33: note = primer
  source 1..33: mol_type = other DNA
gacttatcaaaaacaagccactcttcctgtggc

SEQ ID NO: 16 - DNA, 34 bp, synthetic construct
  misc_feature 1..34: note = primer
  source 1..34: mol_type = other DNA
cttgtttttgataagtccatcattcgctggcgtc

SEQ ID NO: 17 - DNA, 36 bp, synthetic construct
  misc_feature 1..36: note = primer
  source 1..36: mol_type = other DNA
tcggtacccggggatccagcaggccttaagggtaag

SEQ ID NO: 18 - DNA, 34 bp, synthetic construct
  misc_feature 1..34: note = primer
  source 1..34: mol_type = other DNA
aggggcgctgtcttacctcggctggtgggccagc

SEQ ID NO: 19 - DNA, 36 bp, synthetic construct
  misc_feature 1..36: note = primer
  source 1..36: mol_type = other DNA
ggtaagacagcgcccctagttcaaggcttgttaatc

SEQ ID NO: 20 - DNA, 37 bp, synthetic construct
  misc_feature 1..37: note = primer
  source 1..37: mol_type = other DNA
tgcaggtcgactctagaaccgttgaactgcttgccag

SEQ ID NO: 21 - DNA, 34 bp, synthetic construct
  misc_feature 1..34: note = primer
  source 1..34: mol_type = other DNA
tcggtacccggggatccttgaccgtgactacacc

SEQ ID NO: 22 - DNA, 34 bp, synthetic construct
  misc_feature 1..34: note = primer
  source 1..34: mol_type = other DNA
gtatcacgggtgcctctttaatgggccggtgtac

SEQ ID NO: 23 - DNA, 34 bp, synthetic construct
  misc_feature 1..34: note = primer
  source 1..34: mol_type = other DNA
agaggcacccgtgatacgcgcactgcgtttgcca

SEQ ID NO: 24 - DNA, 34 bp, synthetic construct
  misc_feature 1..34: note = primer
  source 1..34: mol_type = other DNA
tgcaggtcgactctagaggcttcgtcaattaccg

SEQ ID NO: 25 - protein, 250 aa, synthetic construct
  REGION 1..250: note = gluconate repressor variant
MPPANESPMTNPLGSAPTPAKPLLDSVLDELGQDINSGKVAVGDTFKLMDIGERFGISRTVAREAMRALEQLGLVASSRRIGITVLPQEEWAVFDKSIIRWRLNDEGQREGQLQSLTELRIAIEPIAARSVALHASTAELEKIRALATEMRQLGESGQGASQRFLEADVTFHELILRYCHNEMFAALIPSISAVLVGRTELGLQPDLPAHEALDNHDKLADALLNRDADAAETASRNILNEVRSALGTLN

SEQ ID NO: 26 - protein, 250 aa, synthetic construct
  REGION 1..250: note = gluconate repressor variant
MPPANESPMTNPLGSAPTPAKPLLDSVLDELGQDIISGKVAVGDTFKLMDIGERFGISATVAREAMRALEQLGLVASSRRIGITVLPQEEWAVFDKSIIRWRLNDEGQREGQLQSLTELRIAIEPIAARSVALHASTAELEKIRALATEMRQLGESGQGASQRFLEADVTFHELILRYCHNEMFAALIPSISAVLVGRTELGLQPDLPAHEALDNHDKLADALLNRDADAAETASRNILNEVRSALGTLN

SEQ ID NO: 27 - protein, 250 aa, synthetic construct
  REGION 1..250: note = gluconate repressor variant
MPPANESPMTNPLGSAPTPAKPLLDSVLDELGQDIISGKVAVGDTFKLMDIGERFGISRLVAREAMRALEQLGLVASSRRIGITVLPQEEWAVFDKSIIRWRLNDEGQREGQLQSLTELRIAIEPIAARSVALHASTAELEKIRALATEMRQLGESGQGASQRFLEADVTFHELILRYCHNEMFAALIPSISAVLVGRTELGLQPDLPAHEALDNHDKLADALLNRDADAAETASRNILNEVRSALGTLN

SEQ ID NO: 28 - protein, 250 aa, synthetic construct
  REGION 1..250: note = gluconate repressor variant
MPPANESPMTNPLGSAPTPAKPLLDSVLDELGQDIISGKVAVGDTFKLMDIGERFGISRTVAAEAMRALEQLGLVASSRRIGITVLPQEEWAVFDKSIIRWRLNDEGQREGQLQSLTELRIAIEPIAARSVALHASTAELEKIRALATEMRQLGESGQGASQRFLEADVTFHELILRYCHNEMFAALIPSISAVLVGRTELGLQPDLPAHEALDNHDKLADALLNRDADAAETASRNILNEVRSALGTLN

SEQ ID NO: 29 - protein, 250 aa, synthetic construct
  REGION 1..250: note = gluconate repressor variant
MPPANESPMTNPLGSAPTPAKPLLDSVLDELGQDIISGKVAVGDTFKLMDIGERFGISRTVAREAMRALKQLGLVASSRRIGITVLPQEEWAVFDKSIIRWRLNDEGQREGQLQSLTELRIAIEPIAARSVALHASTAELEKIRALATEMRQLGESGQGASQRFLEADVTFHELILRYCHNEMFAALIPSISAVLVGRTELGLQPDLPAHEALDNHDKLADALLNRDADAAETASRNILNEVRSALGTLN

SEQ ID NO: 30 - protein, 250 aa, synthetic construct
  REGION 1..250: note = gluconate repressor variant
MPPANESPMTNPLGSAPTPAKPLLDSVLDELGQDIISGKVAVGDTFKLMDIGERFGISRTVAREAMRALEQLGLVASSARIGITVLPQEEWAVFDKSIIRWRLNDEGQREGQLQSLTELRIAIEPIAARSVALHASTAELEKIRALATEMRQLGESGQGASQRFLEADVTFHELILRYCHNEMFAALIPSISAVLVGRTELGLQPDLPAHEALDNHDKLADALLNRDADAAETASRNILNEVRSALGTLN

SEQ ID NO: 31 - protein, 250 aa, synthetic construct
  REGION 1..250: note = gluconate repressor variant
MPPANESPMTNPLGSAPTPAKPLLDSVLDELGQDIISGKVAVGDTFKLMDIGERFGISRTVAREAMRALEQLGLVASSRRIGITVLPQEEWLVFDKSIIRWRLNDEGQREGQLQSLTELRIAIEPIAARSVALHASTAELEKIRALATEMRQLGESGQGASQRFLEADVTFHELILRYCHNEMFAALIPSISAVLVGRTELGLQPDLPAHEALDNHDKLADALLNRDADAAETASRNILNEVRSALGTLN

SEQ ID NO: 32 - DNA, 753 bp, synthetic construct
  misc_feature 1..753: note = gluconate repressor variant
  source 1..753: mol_type = other DNA
atgcccccagcaaacgaaagtcctatgactaatccattaggttctgcccccaccccagccaagccacttcttgacagtgttcttgatgagctcggtcaagatatcaacagtggcaaggttgctgtcggagataccttcaagctgatggacatcggcgagcgttttggtatttcccgcacagtggcacgcgaagcaatgcgcgctttggagcagctcggtcttgtcgcttcttcacgtcgcattggcattactgttttgccacaggaagagtgggctgtttttgataagtccatcattcgctggcgtctcaatgacgaaggtcagcgtgaaggccagcttcagtctcttaccgagcttcgtattgctattgaaccgattgccgcgcgcagcgttgctcttcacgcgtcaaccgccgagctcgagaaaatccgcgcgctggcaacagagatgcgtcagttgggtgaatctggtcagggtgcgtcccagcgcttcctcgaagcggacgtcaccttccacgagctcatcttgcgttattgccacaatgagatgttcgctgcactgattccgtcgattagcgcggttcttgtcggccgcaccgagctcggcctgcagcctgatctgccggcgcacgaggcgctagacaaccacgataagcttgccgacgccctccttaaccgcgacgccgacgccgcagaaactgcgtcccgaaacatcctcaatgaggtgcgcagcgcgctgggcacgctgaactaa

SEQ ID NO: 33 - DNA, 753 bp, synthetic construct
  misc_feature 1..753: note = gluconate repressor variant
  source 1..753: mol_type = other DNA
atgcccccagcaaacgaaagtcctatgactaatccattaggttctgcccccaccccagccaagccacttcttgacagtgttcttgatgagctcggtcaagatatcatcagtggcaaggttgctgtcggagataccttcaagctgatggacatcggcgagcgttttggtatttccgccacagtggcacgcgaagcaatgcgcgctttggagcagctcggtcttgtcgcttcttcacgtcgcattggcattactgttttgccacaggaagagtgggctgtttttgataagtccatcattcgctggcgtctcaatgacgaaggtcagcgtgaaggccagcttcagtctcttaccgagcttcgtattgctattgaaccgattgccgcgcgcagcgttgctcttcacgcgtcaaccgccgagctcgagaaaatccgcgcgctggcaacagagatgcgtcagttgggtgaatctggtcagggtgcgtcccagcgcttcctcgaagcggacgtcaccttccacgagctcatcttgcgttattgccacaatgagatgttcgctgcactgattccgtcgattagcgcggttcttgtcggccgcaccgagctcggcctgcagcctgatctgccggcgcacgaggcgctagacaaccacgataagcttgccgacgccctccttaaccgcgacgccgacgccgcagaaactgcgtcccgaaacatcctcaatgaggtgcgcagcgcgctgggcacgctgaactaa

SEQ ID NO: 34 - DNA, 753 bp, synthetic construct
  misc_feature 1..753: note = gluconate repressor variant
  source 1..753: mol_type = other DNA
atgcccccagcaaacgaaagtcctatgactaatccattaggttctgcccccaccccagccaagccacttcttgacagtgttcttgatgagctcggtcaagatatcatcagtggcaaggttgctgtcggagataccttcaagctgatggacatcggcgagcgttttggtatttcccgcctagtggcacgcgaagcaatgcgcgctttggagcagctcggtcttgtcgcttcttcacgtcgcattggcattactgttttgccacaggaagagtgggctgtttttgataagtccatcattcgctggcgtctcaatgacgaaggtcagcgtgaaggccagcttcagtctcttaccgagcttcgtattgctattgaaccgattgccgcgcgcagcgttgctcttcacgcgtcaaccgccgagctcgagaaaatccgcgcgctggcaacagagatgcgtcagttgggtgaatctggtcagggtgcgtcccagcgcttcctcgaagcggacgtcaccttccacgagctcatcttgcgttattgccacaatgagatgttcgctgcactgattccgtcgattagcgcggttcttgtcggccgcaccgagctcggcctgcagcctgatctgccggcgcacgaggcgctagacaaccacgataagcttgccgacgccctccttaaccgcgacgccgacgccgcagaaactgcgtcccgaaacatcctcaatgaggtgcgcagcgcgctgggcacgctgaactaa

SEQ ID NO: 35 - DNA, 753 bp, synthetic construct
  misc_feature 1..753: note = gluconate repressor variant
  source 1..753: mol_type = other DNA
atgcccccagcaaacgaaagtcctatgactaatccattaggttctgcccccaccccagccaagccacttcttgacagtgttcttgatgagctcggtcaagatatcatcagtggcaaggttgctgtcggagataccttcaagctgatggacatcggcgagcgttttggtatttcccgcacagtggcagccgaagcaatgcgcgctttggagcagctcggtcttgtcgcttcttcacgtcgcattggcattactgttttgccacaggaagagtgggctgtttttgataagtccatcattcgctggcgtctcaatgacgaaggtcagcgtgaaggccagcttcagtctcttaccgagcttcgtattgctattgaaccgattgccgcgcgcagcgttgctcttcacgcgtcaaccgccgagctcgagaaaatccgcgcgctggcaacagagatgcgtcagttgggtgaatctggtcagggtgcgtcccagcgcttcctcgaagcggacgtcaccttccacgagctcatcttgcgttattgccacaatgagatgttcgctgcactgattccgtcgattagcgcggttcttgtcggccgcaccgagctcggcctgcagcctgatctgccggcgcacgaggcgctagacaaccacgataagcttgccgacgccctccttaaccgcgacgccgacgccgcagaaactgcgtcccgaaacatcctcaatgaggtgcgcagcgcgctgggcacgctgaactaa

SEQ ID NO: 36 - DNA, 753 bp, synthetic construct
  misc_feature 1..753: note = gluconate repressor variant
  source 1..753: mol_type = other DNA
atgcccccagcaaacgaaagtcctatgactaatccattaggttctgcccccaccccagccaagccacttcttgacagtgttcttgatgagctcggtcaagatatcatcagtggcaaggttgctgtcggagataccttcaagctgatggacatcggcgagcgttttggtatttcccgcacagtggcacgcgaagcaatgcgcgctttgaagcagctcggtcttgtcgcttcttcacgtcgcattggcattactgttttgccacaggaagagtgggctgtttttgataagtccatcattcgctggcgtctcaatgacgaaggtcagcgtgaaggccagcttcagtctcttaccgagcttcgtattgctattgaaccgattgccgcgcgcagcgttgctcttcacgcgtcaaccgccgagctcgagaaaatccgcgcgctggcaacagagatgcgtcagttgggtgaatctggtcagggtgcgtcccagcgcttcctcgaagcggacgtcaccttccacgagctcatcttgcgttattgccacaatgagatgttcgctgcactgattccgtcgattagcgcggttcttgtcggccgcaccgagctcggcctgcagcctgatctgccggcgcacgaggcgctagacaaccacgataagcttgccgacgccctccttaaccgcgacgccgacgccgcagaaactgcgtcccgaaacatcctcaatgaggtgcgcagcgcgctgggcacgctgaactaa

SEQ ID NO: 37 - DNA, 753 bp, synthetic construct
  misc_feature 1..753: note = gluconate repressor variant
  source 1..753: mol_type = other DNA
atgcccccagcaaacgaaagtcctatgactaatccattaggttctgcccccaccccagccaagccacttcttgacagtgttcttgatgagctcggtcaagatatcatcagtggcaaggttgctgtcggagataccttcaagctgatggacatcggcgagcgttttggtatttcccgcacagtggcacgcgaagcaatgcgcgctttggagcagctcggtcttgtcgcttcttcagctcgcattggcattactgttttgccacaggaagagtgggctgtttttgataagtccatcattcgctggcgtctcaatgacgaaggtcagcgtgaaggccagcttcagtctcttaccgagcttcgtattgctattgaaccgattgccgcgcgcagcgttgctcttcacgcgtcaaccgccgagctcgagaaaatccgcgcgctggcaacagagatgcgtcagttgggtgaatctggtcagggtgcgtcccagcgcttcctcgaagcggacgtcaccttccacgagctcatcttgcgttattgccacaatgagatgttcgctgcactgattccgtcgattagcgcggttcttgtcggccgcaccgagctcggcctgcagcctgatctgccggcgcacgaggcgctagacaaccacgataagcttgccgacgccctccttaaccgcgacgccgacgccgcagaaactgcgtcccgaaacatcctcaatgaggtgcgcagcgcgctgggcacgctgaactaa

SEQ ID NO: 38 - DNA, 753 bp, synthetic construct
  misc_feature 1..753: note = gluconate repressor variant
  source 1..753: mol_type = other DNA
atgcccccagcaaacgaaagtcctatgactaatccattaggttctgcccccaccccagccaagccacttcttgacagtgttcttgatgagctcggtcaagatatcatcagtggcaaggttgctgtcggagataccttcaagctgatggacatcggcgagcgttttggtatttcccgcacagtggcacgcgaagcaatgcgcgctttggagcagctcggtcttgtcgcttcttcacgtcgcattggcattactgttttgccacaggaagagtggcttgtttttgataagtccatcattcgctggcgtctcaatgacgaaggtcagcgtgaaggccagcttcagtctcttaccgagcttcgtattgctattgaaccgattgccgcgcgcagcgttgctcttcacgcgtcaaccgccgagctcgagaaaatccgcgcgctggcaacagagatgcgtcagttgggtgaatctggtcagggtgcgtcccagcgcttcctcgaagcggacgtcaccttccacgagctcatcttgcgttattgccacaatgagatgttcgctgcactgattccgtcgattagcgcggttcttgtcggccgcaccgagctcggcctgcagcctgatctgccggcgcacgaggcgctagacaaccacgataagcttgccgacgccctccttaaccgcgacgccgacgccgcagaaactgcgtcccgaaacatcctcaatgaggtgcgcagcgcgctgggcacgctgaactaa